European Patent Specification EP 3 291 821 B1, published February 25, 2026. Title: DENDRITIC CELL IMMUNOTHERAPY. Applicant: BAYLOR COLLEGE OF MEDICINE Decker, William K. Halpert, Matthew. The sequence listing filed with the application follows.

SEQUENCE LISTING (14 sequences)

SEQ ID NO: 1 - protein, 8 aa, Artificial sequence
  Synthetic peptide
SIINFEKL

SEQ ID NO: 2 - protein, 15 aa, Artificial sequence
  Synthetic peptide
RNLLWLTGKNGLYPN

SEQ ID NO: 3 - protein, 8 aa, Artificial sequence
  Synthetic peptide
WLTGKNGL

SEQ ID NO: 4 - protein, 15 aa, Artificial sequence
  Synthetic peptide
ELLVLLENERTLDFH

SEQ ID NO: 5 - protein, 9 aa, Artificial sequence
  Synthetic peptide
VLLENERTL

SEQ ID NO: 6 - protein, 9 aa, Artificial sequence
  Synthetic peptide
MRMATPLLM

SEQ ID NO: 7 - protein, 9 aa, Artificial sequence
  Synthetic peptide
ATPLLMRPM

SEQ ID NO: 8 - protein, 8 aa, Artificial sequence
  Synthetic peptide
WLTMKNML

SEQ ID NO: 9 - protein, 15 aa, Artificial sequence
  Synthetic peptide
RNLLWLTMKNMLYPN

SEQ ID NO: 10 - protein, 16 aa, Artificial sequence
  Synthetic peptide
WRNLLWLTMKNMLYPN

SEQ ID NO: 11 - protein, 16 aa, Artificial sequence
  Synthetic peptide
WRNLLWLTGKNGLYPN

SEQ ID NO: 12 - DNA, 25 bp, Artificial sequence
  Synthetic primer
atggcttgccttggatttcagcggc

SEQ ID NO: 13 - DNA, 27 bp, Artificial sequence
  Synthetic primer
tcaattgatgggaataaaataaggctg

SEQ ID NO: 14 - protein, 24 aa, Artificial sequence
  Synthetic peptide
LPKSAKPVSQMRMATPLLMRPMSM